European Patent Specification EP 3 630 824 B1, published April 22, 2026. Title: BIOPHARMACEUTICAL COMPOSITIONS AND RELATED METHODS. Applicant: GLAXOSMITHKLINE INTELLECTUAL PROPERTY DEVELOPMENT LIMITED. The sequence listing filed with the application follows.

SEQUENCE LISTING (21 sequences)

SEQ ID NO: 1 - protein, 449 aa, Artificial Sequence
  Amino acid sequence identified using molecular biology techniques.
QVTLRESGPALVKPTQTLTLTCTVSGFSLTGSSVHWVRQPPGKGLEWLGVIWASGGTDYNSALMSRLSISKDTSRNQVVLTMTNMDPVDTATYYCARDPPSGLLRLDYWGRGTLVTVSSASTKGPSVFPLAPSSKSTSGGTAALGCLVKDYFPEPVTVSWNSGALTSGVHTFPAVLQSSGLYSLSSVVTVPSSSLGTQTYICNVNHKPSNTKVDKRVEPKSCDKTHTCPPCPAPELLGGPSVFLFPPKPKDTLYITREPEVTCVVVDVSHEDPEVKFNWYVDGVEVHNAKTKPREEQYNSTYRVVSVLTVLHQDWLNGKEYKCKVSNKALPAPIEKTISKAKGQPREPQVYTLPPSREEMTKNQVSLTCLVKGFYPSDIAVEWESNGQPENNYKTTPPVLDSDGSFFLYSKLTVDKSRWQQGNVFSCSVMHEALHNHYTQKSLSLSPGK

SEQ ID NO: 2 - protein, 220 aa, Artificial Sequence
  Amino acid sequence identified using molecular biology techniques.
DIVMTQSPDSLAVSLGERATINCKSSQSLLNSGNQKNYLAWYQQKPGQPPKLLIYGASTRESGVPDRFSGSGSGTDFTLTISSLQAEDVAVYYCQNVHSFPFTFGGGTKLEIKRTVAAPSVFIFPPSDEQLKSGTASVVCLLNNFYPREAKVQWKVDNALQSGNSQESVTEQDSKDSTYSLSSTLTLSKADYEKHKVYACEVTHQGLSSPVTKSFNRGEC

SEQ ID NO: 3 - protein, 119 aa, Artificial Sequence
  Amino acid sequence identified using molecular biology techniques.
QVTLRESGPALVKPTQTLTLTCTVSGFSLTGSSVHWVRQPPGKGLEWLGVIWASGGTDYNSALMSRLSISKDTSRNQVVLTMTNMDPVDTATYYCARDPPSGLLRLDYWGRGTLVTVSS

SEQ ID NO: 4 - protein, 114 aa, Artificial Sequence
  Amino acid sequence identified using molecular biology techniques.
DIVMTQSPDSLAVSLGERATINCKSSQSLLNSGNQKNYLAWYQQKPGQPPKLLIYGASTRESGVPDRFSGSGSGTDFTLTISSLQAEDVAVYYCQNVHSFPFTFGGGTKLEIKR

SEQ ID NO: 5 - protein, 5 aa, Artificial Sequence
  Amino acid sequence identified using molecular biology techniques.
GSSVH

SEQ ID NO: 6 - protein, 16 aa, Artificial Sequence
  Amino acid sequence identified using molecular biology techniques.
VIWASGGTDYNSALMS

SEQ ID NO: 7 - protein, 11 aa, Artificial Sequence
  Amino acid sequence identified using molecular biology techniques.
DPPSGLLRLDY

SEQ ID NO: 8 - protein, 17 aa, Artificial Sequence
  Amino acid sequence identified using molecular biology techniques.
KSSQSLLNSGNQKNYLA

SEQ ID NO: 9 - protein, 7 aa, Artificial Sequence
  Amino acid sequence identified using molecular biology techniques.
GASTRES

SEQ ID NO: 10 - protein, 9 aa, Artificial Sequence
  Amino acid sequence identified using molecular biology techniques.
QNVHSFPFT

SEQ ID NO: 11 - protein, 115 aa, Homo sapien
IPTEIPTSALVKETLALLSTHRTLLIANETLRIPVPVHKNHQLCTEEIFQGIGTLESQTVQGGTVERLFKNLSLIKKYIDGQKKKCGEERRRVNQFLDYLQEFLGVMNTEWIIES

SEQ ID NO: 12 - protein, 400 aa, Homo sapien
DLLPDEKISLLPPVNFTIKVTGLAQVLLQWKPNPDQEQRNVNLEYQVKINAPKEDDYETRITESKCVTILHKGFSASVRTILQNDHSLLASSWASAELHAPPGSPGTSIVNLTCTTNTTEDNYSRLRSYQVSLHCTWLVGTDAPEDTQYFLYYRYGSWTEECQEYSKDTLGRNIACWFPRTFILSKGRDWLAVLVNGSSKHSAIRPFDQLFALHAIDQINPPLNVTAEIEGTRLSIQWEKPVSAFPIHCFDYEVKIHNTRNGYLQIEKLMTNAFISIIDDLSKYDVQVRAAVSSMCREAGLWSEWSQPIYVGNDEHKPLREWFVIVIMATICFILLILSLICKICHLWIKLFPPIPAPKSNIKDLFVTTNYEKAGSSETEIEVICYIEKPGVETLEDSVF

SEQ ID NO: 13 - DNA, 1404 bp, Artificial Sequence
  Nucleic acid sequence identified using molecular biology techniques.
atgggctggtcctgcatcatcctgtttctggtggccaccgccaccggtgtgcacagccaggtgaccctgagggagagcggccccgccctggtgaagcccacacagaccctcactctgacctgcaccgtgagcggcttcagcctgaccggctctagcgtccactgggtgaggcagccccccggcaagggcctggagtggctgggcgtgatctgggcaagcggggggacggactacaactcggccctgatgagcaggctctccatcagcaaggacaccagccggaaccaggtggtgctgaccatgaccaacatggaccccgtggacaccgccacctattactgcgccagggaccctccctccggcctgctgaggctggactactggggcaggggaacactagtgaccgtgtccagcgccagcaccaagggccccagcgtgttccccctggcccccagcagcaagagcaccagcggcggcacagccgccctgggctgcctggtgaaggactacttccccgagcccgtgaccgtgtcctggaacagcggagccctgaccagcggcgtgcacaccttccccgccgtgctgcagagcagcggcctgtacagcctgagcagcgtggtgaccgtgcccagcagcagcctgggcacccagacctacatctgtaacgtgaaccacaagcccagcaacaccaaggtggacaagcgggtggagcccaagagctgtgacaagacccacacctgccccccctgccctgcccccgagctgctgggaggccccagcgtgttcctgttcccccccaagcctaaggacaccctgtacatcaccagagaacccgaggtgacctgtgtggtggtggatgtgagccacgaggaccctgaggtgaagttcaactggtacgtggacggcgtggaggtgcacaatgccaagaccaagcccagggaggagcagtacaacagcacctaccgggtggtgtccgtgctgaccgtgctgcaccaggattggctgaacggcaaggagtacaagtgtaaggtgtccaacaaggccctgcctgcccctatcgagaaaaccatcagcaaggccaagggccagcccagagagccccaggtgtacaccctgccccctagcagagaggagatgaccaagaaccaggtgtccctgacctgcctggtgaagggcttctaccccagcgacatcgccgtggagtgggagagcaacggccagcccgagaacaactacaagaccaccccccctgtgctggacagcgatggcagcttcttcctgtacagcaagctgaccgtggacaagagcagatggcagcagggcaacgtgttcagctgctccgtgatgcacgaggccctgcacaatcactacacccagaagagcctgagcctgtcccctggcaag

SEQ ID NO: 14 - DNA, 717 bp, Artificial Sequence
  Nucleic acid sequence identified using molecular biology techniques.
atgggctggtcctgcatcatcctgtttctggtggccaccgccaccggtgtgcacagcgacatcgtgatgacccagtctcccgattcactggccgtgagcctgggcgagagggccaccatcaactgcaagagcagccagagcctcctgaacagcggcaaccagaagaactacctggcctggtaccagcagaaacccggccagccccccaagctgctgatctatggcgcctccaccagggagagcggcgtgccagacaggtttagcggcagcggcagcggcaccgacttcaccctgacaatcagcagcctgcaggccgaggacgtggccgtgtactactgccagaacgtccacagcttccccttcaccttcggcgggggaaccaagctggagatcaagcgtacggtggccgcccccagcgtgttcatcttcccccccagcgatgagcagctgaagagcggcaccgccagcgtggtgtgtctgctgaacaacttctacccccgggaggccaaggtgcagtggaaggtggacaatgccctgcagagcggcaacagccaggagagcgtgaccgagcaggacagcaaggactccacctacagcctgagcagcaccctgaccctgagcaaggccgactacgagaagcacaaggtgtacgcctgtgaggtgacccaccagggcctgtccagccccgtgaccaagagcttcaaccggggcgagtgc

SEQ ID NO: 15 - DNA, 356 bp, Artificial Sequence
  Nucleic acid sequence identified using molecular biology techniques.
aggtgaccctgagggagagcggccccgccctggtgaagcccacacagaccctcactctgacctgcaccgtgagcggcttcagcctgaccggctctagcgtccactgggtgaggcagccccccggcaagggcctggagtggctgggcgtgatctgggcaagcggggggacggactacaactcggccctgatgagcaggctctccatcagcaaggacaccagccggaaccaggtggtgctgaccatgaccaacatggaccccgtggacaccgccacctattactgcgccagggaccctccctccggcctgctgaggctggactactggggcaggggaacactagtgaccgtgtccagc

SEQ ID NO: 16 - DNA, 342 bp, Artificial Sequence
  Nucleic acid sequence identified using molecular biology techniques.
gacatcgtgatgacccagtctcccgattcactggccgtgagcctgggcgagagggccaccatcaactgcaagagcagccagagcctcctgaacagcggcaaccagaagaactacctggcctggtaccagcagaaacccggccagccccccaagctgctgatctatggcgcctccaccagggagagcggcgtgccagacaggtttagcggcagcggcagcggcaccgacttcaccctgacaatcagcagcctgcaggccgaggacgtggccgtgtactactgccagaacgtccacagcttccccttcaccttcggcgggggaaccaagctggagatcaagcgt

SEQ ID NO: 17 - DNA, 1347 bp, Artificial Sequence
  Nucleic acid sequence identified using molecular biology techniques.
caggtgaccctgagggagagcggccccgccctggtgaagcccacacagaccctcactctgacctgcaccgtgagcggcttcagcctgaccggctctagcgtccactgggtgaggcagccccccggcaagggcctggagtggctgggcgtgatctgggcaagcggggggacggactacaactcggccctgatgagcaggctctccatcagcaaggacaccagccggaaccaggtggtgctgaccatgaccaacatggaccccgtggacaccgccacctattactgcgccagggaccctccctccggcctgctgaggctggactactggggcaggggaacactagtgaccgtgtccagcgccagcaccaagggccccagcgtgttccccctggcccccagcagcaagagcaccagcggcggcacagccgccctgggctgcctggtgaaggactacttccccgagcccgtgaccgtgtcctggaacagcggagccctgaccagcggcgtgcacaccttccccgccgtgctgcagagcagcggcctgtacagcctgagcagcgtggtgaccgtgcccagcagcagcctgggcacccagacctacatctgtaacgtgaaccacaagcccagcaacaccaaggtggacaagcgggtggagcccaagagctgtgacaagacccacacctgccccccctgccctgcccccgagctgctgggaggccccagcgtgttcctgttcccccccaagcctaaggacaccctgtacatcaccagagaacccgaggtgacctgtgtggtggtggatgtgagccacgaggaccctgaggtgaagttcaactggtacgtggacggcgtggaggtgcacaatgccaagaccaagcccagggaggagcagtacaacagcacctaccgggtggtgtccgtgctgaccgtgctgcaccaggattggctgaacggcaaggagtacaagtgtaaggtgtccaacaaggccctgcctgcccctatcgagaaaaccatcagcaaggccaagggccagcccagagagccccaggtgtacaccctgccccctagcagagaggagatgaccaagaaccaggtgtccctgacctgcctggtgaagggcttctaccccagcgacatcgccgtggagtgggagagcaacggccagcccgagaacaactacaagaccaccccccctgtgctggacagcgatggcagcttcttcctgtacagcaagctgaccgtggacaagagcagatggcagcagggcaacgtgttcagctgctccgtgatgcacgaggccctgcacaatcactacacccagaagagcctgagcctgtcccctggcaag

SEQ ID NO: 18 - DNA, 660 bp, Artificial Sequence
  Nucleic acid sequence identified using molecular biology techniques.
gacatcgtgatgacccagtctcccgattcactggccgtgagcctgggcgagagggccaccatcaactgcaagagcagccagagcctcctgaacagcggcaaccagaagaactacctggcctggtaccagcagaaacccggccagccccccaagctgctgatctatggcgcctccaccagggagagcggcgtgccagacaggtttagcggcagcggcagcggcaccgacttcaccctgacaatcagcagcctgcaggccgaggacgtggccgtgtactactgccagaacgtccacagcttccccttcaccttcggcgggggaaccaagctggagatcaagcgtacggtggccgcccccagcgtgttcatcttcccccccagcgatgagcagctgaagagcggcaccgccagcgtggtgtgtctgctgaacaacttctacccccgggaggccaaggtgcagtggaaggtggacaatgccctgcagagcggcaacagccaggagagcgtgaccgagcaggacagcaaggactccacctacagcctgagcagcaccctgaccctgagcaaggccgactacgagaagcacaaggtgtacgcctgtgaggtgacccaccagggcctgtccagccccgtgaccaagagcttcaaccggggcgagtgc

SEQ ID NO: 19 - protein, 19 aa, Artificial Sequence
  Amino acid sequence identified using molecular biology techniques.
MGWSCIILFLVATATGVHS

SEQ ID NO: 20 - protein, 19 aa, Artificial Sequence
  Amino acid sequence identified using molecular biology techniques.
MGWSCIILFLVATATGVHS

SEQ ID NO: 21 - protein, 11 aa, Artificial Sequence
  Amino acid sequence identified using molecular biology techniques.
WGRGTLVTVSS